European Patent Specification EP 4 106 793 B1, published March 18, 2026. Title: EGFR INHIBITION TRIGGERS AN ADAPTIVE RESPONSE BY CO-OPTING ANTIVIRAL SIGNALING PATHWAYS IN LUNG CANCER. Applicant: Habib, Amyn. The sequence listing filed with the application follows.

SEQUENCE LISTING (8 sequences)

SEQ ID NO: 1 - DNA, 26 bp, Artificial Sequence
  Synthetic Construct; forward primer
gtgaggaaatacttccaaagaatcac

SEQ ID NO: 2 - DNA, 23 bp, Artificial Sequence
  Synthetic Construct; reverse primer
tctcatgatttctgctctgacaa

SEQ ID NO: 3 - DNA, 20 bp, Artificial Sequence
  Synthetic Construct; forward primer
agctgaagcagttccagaag

SEQ ID NO: 4 - DNA, 20 bp, Artificial Sequence
  Synthetic Construct; reverse primer
agtctcattccagccagtgc

SEQ ID NO: 5 - DNA, 21 bp, Artificial Sequence
  Synthetic Construct; forward primer
gggtaactgacttgaatgtcc

SEQ ID NO: 6 - DNA, 20 bp, Artificial Sequence
  Synthetic Construct; reverse primer
ttttcgcttccctgttttag

SEQ ID NO: 7 - DNA, 21 bp, Artificial Sequence
  Synthetic Construct; forward primer
catgtacgttgctatccaggc

SEQ ID NO: 8 - DNA, 21 bp, Artificial Sequence
  Synthetic Construct; reverse primer
ctccttaatgtcacgcacgat